European Patent Specification EP 3 663 402 B1, published April 1, 2026. Title: Powdery mildew resistance marker of Cucurbita maxima, Powdery mildew resistance Cucurbita maxima, method for producing powdery mildew resistance Cucurbita maxima using the same, and method of adding Powdery mildew resistance to Cucurbita maxima. Applicant: Takii & Co.,Ltd. The sequence listing filed with the application follows.

SEQUENCE LISTING (5 sequences)

SEQ ID NO: 1 - DNA, 94 bp, Cucurbita maxima
cttcatattgttttgtggtacaccataagccaagtacgcctttcagaaaacaaagtagatattatagcctgactgtctatgaagaactaaaaag

SEQ ID NO: 2 - DNA, 88 bp, Cucurbita maxima
acatctgaaaaagttgaagctgttatgtgatggagagattgcagagtggttgaaaacgtttgctccccaccttgccaaacaggtcaaa

SEQ ID NO: 3 - DNA, 67 bp, Cucurbita maxima
gagagtgggcaacaatttccccttgaagaagagctcgtcggcggcggtcattgtgtgattactggga

SEQ ID NO: 4 - DNA, 73 bp, Cucurbita maxima
atgaggaatgattacgtttggaaactttgcaggttgtgggagtgctggttggcaagcccctgaacaacttctt

SEQ ID NO: 5 - DNA, 120 bp, Cucurbita maxima
attgtcactagaatttggccaaacactaagtacctggatgtgattgtgaccggagccatggctcagtacatacccaccttggaactttacagtggagggttacccatggcttgcactatg